European Patent Application EP 4 763 220 A2, published June 24, 2026. Title: ANTIGEN RECOGNIZING RECEPTORS TARGETING UPAR AND USES THEREOF. Applicant: MEMORIAL SLOAN-KETTERING CANCER CENTER. Application EP. The sequence listing filed with the application follows.

SEQUENCE LISTING (136 sequences)

SEQ ID NO: 1 - protein, 8 aa, synthetic construct
  REGION 1..8: note = Synthetic
GFTFSDDY

SEQ ID NO: 2 - protein, 8 aa, synthetic construct
  REGION 1..8: note = Synthetic
ISGSGGST

SEQ ID NO: 3 - protein, 21 aa, synthetic construct
  REGION 1..21: note = Synthetic
ATGVPYCSTTRCPPYYYTMDV

SEQ ID NO: 4 - protein, 7 aa, synthetic construct
  REGION 1..7: note = Synthetic
QSVDSTA

SEQ ID NO: 5 - skipped

SEQ ID NO: 6 - protein, 9 aa, synthetic construct
  REGION 1..9: note = Synthetic
QQDGEYPLT

SEQ ID NO: 7 - protein, 128 aa, synthetic construct
  REGION 1..128: note = Synthetic
EVQLLESGGGLVQPGGSLRLSCAASGFTFSDDYMSWVRQAPGKGLEWVSVISGSGGSTDYADSVKGRFTISRDNSKNTLYLQMNSLRAEDTAVYYCATGVPYCSTTRCPPYYYTMDVWGQGTTVTVSS

SEQ ID NO: 8 - protein, 108 aa, synthetic construct
  REGION 1..108: note = Synthetic
EIVLTQSPGTLSLSPGERATLSCRASQSVDSTALAWYQQKPGQAPRLLIYAASSRATGIPDRFSGSGSGTDFTLTISRLEPEDFAVYYCQQDGEYPLTFGQGTKVEIK

SEQ ID NO: 9 - protein, 255 aa, synthetic construct
  REGION 1..255: note = Synthetic
EIVLTQSPGTLSLSPGERATLSCRASQSVDSTALAWYQQKPGQAPRLLIYAASSRATGIPDRFSGSGSGTDFTLTISRLEPEDFAVYYCQQDGEYPLTFGQGTKVEIKGGGGSGGGGSGGGSGGGGSEVQLLESGGGLVQPGGSLRLSCAASGFTFSDDYMSWVRQAPGKGLEWVSVISGSGGSTDYADSVKGRFTISRDNSKNTLYLQMNSLRAEDTAVYYCATGVPYCSTTRCPPYYYTMDVWGQGTTVTVSS

SEQ ID NO: 10 - protein, 765 aa, synthetic construct
  REGION 1..765: note = Synthetic
GAAATTGTGTTGACGCAGTCTCCAGGCACCCTGTCTTTGTCTCCAGGGGAACGTGCCACCCTCTCCTGCCGTGCCAGTCAGAGTGTTGACAGCACCGCCTTAGCCTGGTATCAGCAGAAACCTGGCCAGGCTCCCCGACTCCTCATCTATGCCGCATCTAGCCGTGCCACTGGTATCCCAGACCGTTTCAGTGGCAGTGGGTCTGGGACAGACTTCACTCTCACCATCAGCAGACTGGAGCCTGAAGATTTTGCAGTGTATTACTGTCAGCAGGACGGCGAGTATCCTCTGACGTTCGGCCAAGGTACCAAGGTGGAAATCAAAGGTGGTGGTGGTTCAGGTGGTGGTGGTTCTGGCGGCGGCTCCGGTGGTGGTGGATCCGAGGTGCAGCTGTTGGAGTCTGGGGGAGGCTTGGTACAGCCTGGGGGGTCCCTGCGACTCTCCTGTGCAGCCTCTGGATTCACCTTTAGCGACGACTATATGAGCTGGGTCCGCCAGGCTCCAGGGAAGGGGCTGGAGTGGGTGTCAGTGATTAGCGGTAGCGGTGGTAGCACAGACTACGCAGACTCCGTGAAGGGCCGGTTCACCATCTCCCGTGACAATTCCAAGAACACGCTGTATCTGCAAATGAACAGCCTGCGTGCCGAGGACACGGCTGTGTATTACTGTGCGACAGGGGTCCCATATTGTAGTACTACCAGGTGCCCCCCATACTACTACACTATGGACGTCTGGGGCCAAGGGACCACGGTCACTGTCTCNTCA

SEQ ID NO: 11 - protein, 8 aa, synthetic construct
  REGION 1..8: note = Synthetic
GFTFSSDG

SEQ ID NO: 12 - protein, 16 aa, synthetic construct
  REGION 1..16: note = Synthetic
ARETVWDPLSLGAFDI

SEQ ID NO: 13 - protein, 7 aa, synthetic construct
  REGION 1..7: note = Synthetic
QSVQASS

SEQ ID NO: 14 - protein, 9 aa, synthetic construct
  REGION 1..9: note = Synthetic
QQYGSSPIT

SEQ ID NO: 15 - protein, 123 aa, synthetic construct
  REGION 1..123: note = Synthetic
EVQLLESGGGLVQPGGSLRLSCAASGFTFSSDGMSWVRQAPGKGLEWVSAISGSGGSTNYADSVKGRFTISRDNSKNTLYLQMNSLRAEDTAVYYCARETVWDPLSLGAFDIWGQGTMVTVSS

SEQ ID NO: 16 - protein, 108 aa, synthetic construct
  REGION 1..108: note = Synthetic
EIVLTQSPGTLSLSPGERATLSCRASQSVQASSLAWYQQKPGQAPRLLIYAASSRATGIPDRFSGSGSGTDFTLTISRLEPEDFAVYYCQQYGSSPITFGQGTKVEIK

SEQ ID NO: 17 - protein, 250 aa, synthetic construct
  REGION 1..250: note = Synthetic
EIVLTQSPGTLSLSPGERATLSCRASQSVQASSLAWYQQKPGQAPRLLIYAASSRATGIPDRFSGSGSGTDFTLTISRLEPEDFAVYYCQQYGSSPITFGQGTKVEIKGGGGSGGGGSGGGSGGGGSEVQLLESGGGLVQPGGSLRLSCAASGFTFSSDGMSWVRQAPGKGLEWVSAISGSGGSTNYADSVKGRFTISRDNSKNTLYLQMNSLRAEDTAVYYCARETVWDPLSLGAFDIWGQGTMVTVSS

SEQ ID NO: 18 - DNA, 750 bp, synthetic construct
  misc_feature 1..750: note = Synthetic
  source 1..750: mol_type = other DNA
gaaattgtgttgacgcagtctccaggcaccctgtctttgtctccaggggaacgtgccaccctctcctgccgtgccagtcagagtgttcaggccagcagcttagcctggtatcagcagaaacctggccaggctccccgactcctcatctatgccgcatctagccgtgccactggtatcccagaccgtttcagtggcagtgggtctgggacagacttcactctcaccatcagcagactggagcctgaagattttgcagtgtattactgtcagcagtatggcagcagccctatcacgttcggccaaggtaccaaggtggaaatcaaaggtggtggtggttcaggtggtggtggttctggcggcggctccggtggtggtggatccgaggtgcagctgttggagtctgggggaggcttggtacagcctggggggtccctgcgactctcctgtgcagcctctggattcacctttagcagcgacggcatgagctgggtccgccaggctccagggaaggggctggagtgggtgtcagccattagcggtagcggtggtagcacaaattacgcagactccgtgaagggccggttcaccatctcccgtgacaattccaagaacacgctgtatctgcaaatgaacagcctgcgtgccgaggacacggccgtgtattactgtgcgagagagacggtgtgggatcccctatccctgggtgcttttgatatctggggccaagggacaatggtcaccgtctcttca

SEQ ID NO: 19 - protein, 8 aa, synthetic construct
  REGION 1..8: note = Synthetic
GFTFTDYY

SEQ ID NO: 20 - protein, 12 aa, synthetic construct
  REGION 1..12: note = Synthetic
ARDWGGSIPLDI

SEQ ID NO: 21 - protein, 7 aa, synthetic construct
  REGION 1..7: note = Synthetic
QSVSHSY

SEQ ID NO: 22 - protein, 9 aa, synthetic construct
  REGION 1..9: note = Synthetic
QQYSYSPFT

SEQ ID NO: 23 - protein, 119 aa, synthetic construct
  REGION 1..119: note = Synthetic
EVQLLESGGGLVQPGGSLRLSCAASGFTFTDYYMSWVRQAPGKGLEWVSDISGSGGSTYYADSVKGRFTISRDNSKNTLYLQMNSLRAEDTAVYYCARDWGGSIPLDIWGQGTMVTVSS

SEQ ID NO: 24 - protein, 108 aa, synthetic construct
  REGION 1..108: note = Synthetic
EIVLTQSPGTLSLSPGERATLSCRASQSVSHSYLAWYQQKPGQAPRLLIYAASSRATGIPDRFSGSGSGTDFTLTISRLEPEDFAVYYCQQYSYSPFTFGQGTKVEIK

SEQ ID NO: 25 - protein, 246 aa, synthetic construct
  REGION 1..246: note = Synthetic
EIVLTQSPGTLSLSPGERATLSCRASQSVSHSYLAWYQQKPGQAPRLLIYAASSRATGIPDRFSGSGSGTDFTLTISRLEPEDFAVYYCQQYSYSPFTFGQGTKVEIKGGGGSGGGGSGGGSGGGGSEVQLLESGGGLVQPGGSLRLSCAASGFTFTDYYMSWVRQAPGKGLEWVSDISGSGGSTYYADSVKGRFTISRDNSKNTLYLQMNSLRAEDTAVYYCARDWGGSIPLDIWGQGTMVTVSS

SEQ ID NO: 26 - DNA, 711 bp, synthetic construct
  misc_feature 1..711: note = Synthetic
  source 1..711: mol_type = other DNA
gaaattgtgttgacgcagtctccaggcaccctgtctttgtctccaggggaacgtgccaccctctcctgccgtgccagtcagagtgttagccacagctatttagcctggtatcagcagaaacctggccaggctccccgactcctcatctatgccgcatctagccgtgccactggtatcccagaccgtttcagtggcagtgggtctgggacagacttcactctcaccatcagcagactggagcctgaagattttgcagtgtattactgtcagcagtatagctatagcccttttacgttcggccaaggtaccaaggtggaaatcaaaggtggtggtggttcaggtggtggtggttctgaggtgcagctgttggagtctgggggaggcttggtacagcctggggggtccctgcgactctcctgtgcagcctctggattcacctttaccgactattatatgagctgggtccgccaggctccagggaaggggctggagtgggtgtcagacattagcggtagtggtggtagcacatactacgcagactccgtgaagggccggttcaccatctcccgtgacaattccaagaacacgctgtatctgcaaatgaacagcctgcgtgccgaggacacggccgtgtattactgtgcgagggattgggggggttccatccccctagatatctggggccaagggacaatggtcaccgtctcttca

SEQ ID NO: 27 - protein, 8 aa, synthetic construct
  REGION 1..8: note = Synthetic
ISGRGGQT

SEQ ID NO: 28 - protein, 16 aa, synthetic construct
  REGION 1..16: note = Synthetic
ARDSYLTIWSGEGFDY

SEQ ID NO: 29 - protein, 7 aa, synthetic construct
  REGION 1..7: note = Synthetic
QSVDRSY

SEQ ID NO: 30 - protein, 9 aa, synthetic construct
  REGION 1..9: note = Synthetic
QQDSYSPIT

SEQ ID NO: 31 - protein, 123 aa, synthetic construct
  REGION 1..123: note = Synthetic
EVQLLESGGGLVQPGGSLRLSCAASGFTFTDYYMSWVRQAPGKGLEWVSRISGRGGQTDYADSVKGRFTISRDNSKNTLYLQMNSLRAEDTAVYYCARDSYLTIWSGEGFDYWGQGTLVTVSS

SEQ ID NO: 32 - protein, 108 aa, synthetic construct
  REGION 1..108: note = Synthetic
EIVLTQSPGTLSLSPGERATLSCRASQSVDRSYLAWYQQKPGQAPRLLIYGASSRATGIPDRFSGSGSGTDFTLTISRLEPEDFAVYYCQQDSYSPITFGQGTKVEIK

SEQ ID NO: 33 - protein, 250 aa, synthetic construct
  REGION 1..250: note = Synthetic
EIVLTQSPGTLSLSPGERATLSCRASQSVDRSYLAWYQQKPGQAPRLLIYGASSRATGIPDRFSGSGSGTDFTLTISRLEPEDFAVYYCQQDSYSPITFGQGTKVEIKGGGGSGGGGSGGGSGGGGSEVQLLESGGGLVQPGGSLRLSCAASGFTFTDYYMSWVRQAPGKGLEWVSRISGRGGQTDYADSVKGRFTISRDNSKNTLYLQMNSLRAEDTAVYYCARDSYLTIWSGEGFDYWGQGTLVTVSS

SEQ ID NO: 34 - DNA, 750 bp, synthetic construct
  misc_feature 1..750: note = Synthetic
  source 1..750: mol_type = other DNA
gaaattgtgttgacgcagtctccaggcaccctgtctttgtctccaggggaacgtgccaccctctcctgccgtgccagtcagagtgttgaccgcagctatttagcctggtatcagcagaaacctggccaggctccccgactcctcatctatggcgcatctagccgtgccactggtatcccagaccgtttcagtggcagtgggtctgggacagacttcactctcaccatcagcagactggagcctgaagattttgcagtgtattactgtcagcaggacagctatagccctatcacgttcggccaaggtaccaaggtggaaatcaaaggtggtggtggttcaggtggtggtggttctggcggcggctccggtggtggtggatccgaggtgcagctgttggagtctgggggaggcttggtacagcctggggggtccctgcgactctcctgtgcagcctctggattcacctttaccgactattatatgagctgggtccgccaggctccagggaaggggctggagtgggtgtcacgcattagcggtcgcggtggtcagacagactacgcagactccgtgaagggccggttcaccatctcccgtgacaattccaagaacacgctgtatctgcaaatgaacagcctgcgtgccgaggacacggctgtgtattactgtgcgagagattcttacctcacaatatggtccggggaggggtttgactactggggccagggaaccctggtcaccgtctcctca

SEQ ID NO: 35 - protein, 8 aa, synthetic construct
  REGION 1..8: note = Synthetic
GFTFTSYA

SEQ ID NO: 36 - protein, 10 aa, synthetic construct
  REGION 1..10: note = Synthetic
ISGSGYGGST

SEQ ID NO: 37 - protein, 16 aa, synthetic construct
  REGION 1..16: note = Synthetic
VKDKSHTRVEADAFDI

SEQ ID NO: 38 - protein, 12 aa, synthetic construct
  REGION 1..12: note = Synthetic
QSVLSSNNNENN

SEQ ID NO: 39 - skipped

SEQ ID NO: 40 - protein, 9 aa, synthetic construct
  REGION 1..9: note = Synthetic
QQGTSSPIT

SEQ ID NO: 41 - protein, 125 aa, synthetic construct
  REGION 1..125: note = Synthetic
EVQLLESGGGLVQPGGSLRLSCAASGFTFTSYAMSWVRQAPGKGLEWVSRISGSGYGGSTYYADSVKGRFTISRDNSKNTLYLQMNSLRAEDTAVYYCVKDKSHTRVEADAFDIWGQGTMVTVSS

SEQ ID NO: 42 - protein, 113 aa, synthetic construct
  REGION 1..113: note = Synthetic
DIVMTQSPDSLAVSLGERATINCKSSQSVLSSNNNENNLAWYQQKPGQPPKLLIYDASTRESGVPDRFSGSGSGTDFTLTISSLQAEDVAVYYCQQGTSSPITFGQGTKVEIK

SEQ ID NO: 43 - protein, 257 aa, synthetic construct
  REGION 1..257: note = Synthetic
DIVMTQSPDSLAVSLGERATINCKSSQSVLSSNNNENNLAWYQQKPGQPPKLLIYDASTRESGVPDRFSGSGSGTDFTLTISSLQAEDVAVYYCQQGTSSPITFGQGTKVEIKGGGGSGGGGSGGGSGGGGSEVQLLESGGGLVQPGGSLRLSCAASGFTFTSYAMSWVRQAPGKGLEWVSRISGSGYGGSTYYADSVKGRFTISRDNSKNTLYLQMNSLRAEDTAVYYCVKDKSHTRVEADAFDIWGQGTMVTVSS

SEQ ID NO: 44 - DNA, 771 bp, synthetic construct
  misc_feature 1..771: note = Synthetic
  source 1..771: mol_type = other DNA
gacatcgtgatgacccagtctccagactccctggctgtgtctctgggcgagcgtgccaccatcaactgcaagtccagccagagtgttttaagtagcaataacaatgagaacaatttagcttggtatcagcagaaaccaggacagcctcctaagctgctcatttacgacgcatctacccgggaatccggggtccctgaccgattcagtggcagcgggtctgggacagatttcactctcaccatcagcagcctgcaggctgaagatgtggcagtttattactgtcagcaaggcaccagcagccctatcacgttcggccaaggtaccaaggtggaaatcaaaggtggtggtggttcaggtggtggtggttctggcggcggctccggtggtggtggatccgaggtgcagctgttggagtctgggggaggcttggtacagcctggggggtccctgcgactctcctgtgcagcctctggattcacctttaccagctatgccatgagctgggtccgccaggctccagggaaggggctggagtgggtgtcacgcattagcggtagcggttatggtggtagcacatattacgcagactccgtgaagggccggttcaccatctcccgtgacaattccaagaacacgctgtatctgcaaatgaacagcctgcgtgccgaggacacggctgtgtattactgtgtaaaagataagtcgcatactcgggttgaggcggatgcttttgatatctggggccaagggacaatggtcaccgtctcttca

SEQ ID NO: 45 - protein, 8 aa, synthetic construct
  REGION 1..8: note = Synthetic
GFTFSSYG

SEQ ID NO: 46 - protein, 8 aa, synthetic construct
  REGION 1..8: note = Synthetic
ISGYGSST

SEQ ID NO: 47 - protein, 15 aa, synthetic construct
  REGION 1..15: note = Synthetic
AKDRYSLSYYYGMDV

SEQ ID NO: 48 - protein, 12 aa, synthetic construct
  REGION 1..12: note = Synthetic
QSVLSSSNNYNR

SEQ ID NO: 49 - protein, 9 aa, synthetic construct
  REGION 1..9: note = Synthetic
QQYDSRPIT

SEQ ID NO: 50 - protein, 122 aa, synthetic construct
  REGION 1..122: note = Synthetic
EVQLLESGGGLVQPGGSLRLSCAASGFTFSSYGMSWVRQAPGKGLEWVSDISGYGSSTYYADSVKGRFTISRDNSKNTLYLQMNSLRAEDTAVYYCAKDRYSLSYYYGMDVWGQGTTVTVSS

SEQ ID NO: 51 - protein, 113 aa, synthetic construct
  REGION 1..113: note = Synthetic
DIVMTQSPDSLAVSLGERATINCKSSQSVLSSSNNYNRLAWYQQKPGQPPKLLIYAASTRESGVPDRFSGSGSGTDFTLTISSLQAEDVAVYYCQQYDSRPITFGQGTKVEIK

SEQ ID NO: 52 - protein, 254 aa, synthetic construct
  REGION 1..254: note = Synthetic
DIVMTQSPDSLAVSLGERATINCKSSQSVLSSSNNYNRLAWYQQKPGQPPKLLIYAASTRESGVPDRFSGSGSGTDFTLTISSLQAEDVAVYYCQQYDSRPITFGQGTKVEIKGGGGSGGGGSGGGSGGGGSEVQLLESGGGLVQPGGSLRLSCAASGFTFSSYGMSWVRQAPGKGLEWVSDISGYGSSTYYADSVKGRFTISRDNSKNTLYLQMNSLRAEDTAVYYCAKDRYSLSYYYGMDVWGQGTTVTVSS

SEQ ID NO: 53 - DNA, 762 bp, synthetic construct
  misc_feature 1..762: note = Synthetic
  source 1..762: mol_type = other DNA
gacatcgtgatgacccagtctccagactccctggctgtgtctctgggcgagcgtgccaccatcaactgcaagtccagccagagtgttttaagcagcagcaacaattataaccgcttagcttggtatcagcagaaaccaggacagcctcctaagctgctcatttacgccgcatctacccgggaatccggggtccctgaccgattcagtggcagcgggtctgggacagatttcactctcaccatcagcagcctgcaggctgaagatgtggcagtttattactgtcagcaatatgacagccgccctatcacgttcggccaaggtaccaaggtggaaatcaaaggtggtggtggttcaggtggtggtggttctggcggcggctccggtggtggtggatccgaggtgcagctgttggagtctgggggaggcttggtacagcctggggggtccctgcgactctcctgtgcagcctctggattcacctttagcagctatggcatgagctgggtccgccaggctccagggaaggggctggagtgggtgtcagacattagcggttatggtagcagcacatattacgcagactccgtgaagggccggttcaccatctcccgtgacaattccaagaacacgctgtatctgcaaatgaacagcctgcgtgccgaggacacggctgtgtattactgtgcaaaagaccggtatagcctttcctactactacggtatggacgtctggggccaagggaccacggtcaccgtctcctca

SEQ ID NO: 54 - protein, 8 aa, synthetic construct
  REGION 1..8: note = Synthetic
GFTFTSSA

SEQ ID NO: 55 - protein, 8 aa, synthetic construct
  REGION 1..8: note = Synthetic
IYGGGGST

SEQ ID NO: 56 - protein, 14 aa, synthetic construct
  REGION 1..14: note = Synthetic
ARAVWTSNGYYFDT

SEQ ID NO: 57 - protein, 12 aa, synthetic construct
  REGION 1..12: note = Synthetic
QSVLYSSNNKNN

SEQ ID NO: 58 - protein, 9 aa, synthetic construct
  REGION 1..9: note = Synthetic
QQGYSEPIT

SEQ ID NO: 59 - protein, 121 aa, synthetic construct
  REGION 1..121: note = Synthetic
EVQLLESGGGLVQPGGSLRLSCAASGFTFTSSAMSWVRQAPGKGLEWVSDIYGGGGSTSYADSVKGRFTISRDNSKNTLYLQMNSLRAEDTAVYYCARAVWTSNGYYFDTWGQGTLVTVSS

SEQ ID NO: 60 - protein, 113 aa, synthetic construct
  REGION 1..113: note = Synthetic
DIVMTQSPDSLAVSLGERATINCKSSQSVLYSSNNKNNLAWYQQKPGQPPKLLIYAASTRESGVPDRFSGSGSGTDFTLTISSLQAEDVAVYYCQQGYSEPITFGQGTKVEIK

SEQ ID NO: 61 - protein, 253 aa, synthetic construct
  REGION 1..253: note = Synthetic
DIVMTQSPDSLAVSLGERATINCKSSQSVLYSSNNKNNLAWYQQKPGQPPKLLIYAASTRESGVPDRFSGSGSGTDFTLTISSLQAEDVAVYYCQQGYSEPITFGQGTKVEIKGGGGSGGGGSGGGSGGGGSEVQLLESGGGLVQPGGSLRLSCAASGFTFTSSAMSWVRQAPGKGLEWVSDIYGGGGSTSYADSVKGRFTISRDNSKNTLYLQMNSLRAEDTAVYYCARAVWTSNGYYFDTWGQGTLVTVSS

SEQ ID NO: 62 - DNA, 759 bp, synthetic construct
  misc_feature 1..759: note = Synthetic
  source 1..759: mol_type = other DNA
gacatcgtgatgacccagtctccagactccctggctgtgtctctgggcgagcgtgccaccatcaactgcaagtccagccagagtgttttatatagcagcaacaataaaaacaatttagcttggtatcagcagaaaccaggacagcctcctaagctgctcatttacgccgcatctacccgggaatccggggtccctgaccgattcagtggcagcgggtctgggacagatttcactctcaccatcagcagcctgcaggctgaagatgtggcagtttattactgtcagcaaggctatagcgaacctatcacgttcggccaaggtaccaaggtggaaatcaaaggtggtggtggttcaggtggtggtggttctggcggcggctccggtggtggtggatccgaggtgcagctgttggagtctgggggaggcttggtacagcctggggggtccctgcgactctcctgtgcagcctctggattcacctttaccagcagcgccatgagctgggtccgccaggctccagggaaggggctggagtgggtgtcagacatttatggtggcggtggtagcacaagctacgcagactccgtgaagggccggttcaccatctcccgtgacaattccaagaacacgctgtatctgcaaatgaacagcctgcgtgccgaggacacggctgtgtattactgtgcaagagccgtctggacgagtaatggttattacttcgacacctggggccagggaaccctggtcaccgtctcctca

SEQ ID NO: 63 - protein, 8 aa, synthetic construct
  REGION 1..8: note = Synthetic
GFTFSDYA

SEQ ID NO: 64 - protein, 8 aa, synthetic construct
  REGION 1..8: note = Synthetic
IQGGGGYT

SEQ ID NO: 65 - protein, 24 aa, synthetic construct
  REGION 1..24: note = Synthetic
AKDQLEHYDFWSGYLNYYYYGMDV

SEQ ID NO: 66 - protein, 7 aa, synthetic construct
  REGION 1..7: note = Synthetic
QSVSSSY

SEQ ID NO: 67 - skipped

SEQ ID NO: 68 - protein, 9 aa, synthetic construct
  REGION 1..9: note = Synthetic
QQYSRSPLT

SEQ ID NO: 69 - protein, 131 aa, synthetic construct
  REGION 1..131: note = Synthetic
EVQLLESGGGLVQPGGSLRLSCAASGFTFSDYAMSWVRQAPGKGLEWVSEIQGGGGYTNYADSVKGRFTISRDNSKNTLYLQMNSLRAEDTAVYYCAKDQLEHYDFWSGYLNYYYYGMDVWGQGTTVTVSS

SEQ ID NO: 70 - protein, 108 aa, synthetic construct
  REGION 1..108: note = Synthetic
EIVLTQSPGTLSLSPGERATLSCRASQSVSSSYLAWYQQKPGQAPRLLIYGASSRATGIPDRFSGSGSGTDFTLTISRLEPEDFAVYYCQQYSRSPLTFGQGTKVEIK

SEQ ID NO: 71 - protein, 258 aa, synthetic construct
  REGION 1..258: note = Synthetic
EIVLTQSPGTLSLSPGERATLSCRASQSVSSSYLAWYQQKPGQAPRLLIYGASSRATGIPDRFSGSGSGTDFTLTISRLEPEDFAVYYCQQYSRSPLTFGQGTKVEIKGGGGSGGGGSGGGSGGGGSEVQLLESGGGLVQPGGSLRLSCAASGFTFSDYAMSWVRQAPGKGLEWVSEIQGGGGYTNYADSVKGRFTISRDNSKNTLYLQMNSLRAEDTAVYYCAKDQLEHYDFWSGYLNYYYYGMDVWGQGTTVTVSS

SEQ ID NO: 72 - DNA, 774 bp, synthetic construct
  misc_feature 1..774: note = Synthetic
  source 1..774: mol_type = other DNA
gaaattgtgttgacgcagtctccaggcaccctgtctttgtctccaggggaacgtgccaccctctcctgccgtgccagtcagagtgttagcagcagctatttagcctggtatcagcagaaacctggccaggctccccgactcctcatctatggcgcatctagccgtgccactggtatcccagaccgtttcagtggcagtgggtctgggacagacttcactctcaccatcagcagactggagcctgaagattttgcagtgtattactgtcagcagtatagccgcagccctctgacgttcggccaaggtaccaaggtggaaatcaaaggtggtggtggttcaggtggtggtggttctggcggcggctccggtggtggtggatccgaggtgcagctgttggagtctgggggaggcttggtacagcctggggggtccctgcgactctcctgtgcagcctctggattcacctttagcgactatgccatgagctgggtccgccaggctccagggaaggggctggagtgggtgtcagagattcagggtggcggtggttatacaaattacgcagactccgtgaagggccggttcaccatctcccgtgacaattccaagaacacgctgtatctgcaaatgaacagcctgcgtgccgaggacacggccgtgtattactgtgcgaaagatcaattagagcattacgatttttggagtggttacctgaactactactactacggtatggacgtctggggccaagggaccacggtcaccgtctcctca

SEQ ID NO: 73 - protein, 8 aa, synthetic construct
  REGION 1..8: note = Synthetic
GFTFSSYA

SEQ ID NO: 74 - protein, 8 aa, synthetic construct
  REGION 1..8: note = Synthetic
ISGSGGDT

SEQ ID NO: 75 - protein, 24 aa, synthetic construct
  REGION 1..24: note = Synthetic
ANRDTRLYYDFWSGYWNAPHAFDI

SEQ ID NO: 76 - protein, 7 aa, synthetic construct
  REGION 1..7: note = Synthetic
QSVSSTS

SEQ ID NO: 77 - protein, 9 aa, synthetic construct
  REGION 1..9: note = Synthetic
QQYSEYPLT

SEQ ID NO: 78 - protein, 131 aa, synthetic construct
  REGION 1..131: note = Synthetic
EVQLLESGGGLVQPGGSLRLSCAASGFTFSSYAMSWVRQAPGKGLEWVSEISGSGGDTKYADSVKGRFTISRDNSKNTLYLQMNSLRAEDTAVYYCANRDTRLYYDFWSGYWNAPHAFDIWGQGTMVTVSS

SEQ ID NO: 79 - protein, 108 aa, synthetic construct
  REGION 1..108: note = Synthetic
EIVLTQSPGTLSLSPGERATLSCRASQSVSSTSLAWYQQKPGQAPRLLIYGASSRATGIPDRFSGSGSGTDFTLTISRLEPEDFAVYYCQQYSEYPLTFGQGTKVEIK

SEQ ID NO: 80 - protein, 258 aa, synthetic construct
  REGION 1..258: note = Synthetic
EIVLTQSPGTLSLSPGERATLSCRASQSVSSTSLAWYQQKPGQAPRLLIYGASSRATGIPDRFSGSGSGTDFTLTISRLEPEDFAVYYCQQYSEYPLTFGQGTKVEIKGGGGSGGGGSGGGSGGGGSEVQLLESGGGLVQPGGSLRLSCAASGFTFSSYAMSWVRQAPGKGLEWVSEISGSGGDTKYADSVKGRFTISRDNSKNTLYLQMNSLRAEDTAVYYCANRDTRLYYDFWSGYWNAPHAFDIWGQGTMVTVSS

SEQ ID NO: 81 - DNA, 775 bp, synthetic construct
  misc_feature 1..775: note = Synthetic
  source 1..775: mol_type = other DNA
gaaattgtgttgacgcagtctccaggcaccctgtctttgtctccaggggaacgtgccaccctctcctgccgtgccagtcagagtgttagcagcaccagcttagcctggtatcagcagaaacctggccaggctccccgactcctcatctatggcgcatctagccgtgccactggtatcccagaccgtttcagtggcagtgggtctgggacagacttcactctcaccatcagcagactggagcctgaagattttgcagtgtattactgtcagcagtatagcgagtatcctctgacgttcggccaaggtaccaaggtggaaatcaaaggtggtggtggttcaggtggtggtggttctggcggcggctccggtggtggtggatccgaggtgcagctgttggagtctgggggaggcttggtacagcctggggggtccctgcgactctcctgtgcagcctctggattcacctttagcagctatgccatgagctgggtccgccaggctccagggaaggggctggagtgggtgtcagagattagcggtagcggtggtgacacaaaatacgcagactccgtgaagggccggttcaccatctcccgtgacaattccaagaacacgctgtatctgcaaatgaacagcctgcgtgccgaggacacggccgtgtattactgtgcgaaccgcgacacgcgcctttattacgatttttggagtggttattggaatgccccccatgcttttgatatctggggccaagggacaatggtcaccgtctcttcag

SEQ ID NO: 82 - protein, 8 aa, synthetic construct
  REGION 1..8: note = Synthetic
ISGSGGQT

SEQ ID NO: 83 - protein, 16 aa, synthetic construct
  REGION 1..16: note = Synthetic
ARDRTMGSYYYYGMDV

SEQ ID NO: 84 - protein, 7 aa, synthetic construct
  REGION 1..7: note = Synthetic
QSVSSNS

SEQ ID NO: 85 - protein, 9 aa, synthetic construct
  REGION 1..9: note = Synthetic
QQYEQSPIT

SEQ ID NO: 86 - protein, 123 aa, synthetic construct
  REGION 1..123: note = Synthetic
EVQLLESGGGLVQPGGSLRLSCAASGFTFSSYGMSWVRQAPGKGLEWVSAISGSGGQTNYADSVKGRFTISRDNSKNTLYLQMNSLRAEDTAVYYCARDRTMGSYYYYGMDVWGQGTTVTVSS

SEQ ID NO: 87 - protein, 108 aa, synthetic construct
  REGION 1..108: note = Synthetic
EIVLTQSPGTLSLSPGERATLSCRASQSVSSNSLAWYQQKPGQAPRLLIYGASSRATGIPDRFSGSGSGTDFTLTISRLEPEDFAVYYCQQYEQSPITFGQGTKVEIK

SEQ ID NO: 88 - protein, 250 aa, synthetic construct
  REGION 1..250: note = Synthetic
EIVLTQSPGTLSLSPGERATLSCRASQSVSSNSLAWYQQKPGQAPRLLIYGASSRATGIPDRFSGSGSGTDFTLTISRLEPEDFAVYYCQQYEQSPITFGQGTKVEIKGGGGSGGGGSGGGSGGGGSEVQLLESGGGLVQPGGSLRLSCAASGFTFSSYGMSWVRQAPGKGLEWVSAISGSGGQTNYADSVKGRFTISRDNSKNTLYLQMNSLRAEDTAVYYCARDRTMGSYYYYGMDVWGQGTTVTVSS

SEQ ID NO: 89 - DNA, 750 bp, synthetic construct
  misc_feature 1..750: note = Synthetic
  source 1..750: mol_type = other DNA
gaaattgtgttgacgcagtctccaggcaccctgtctttgtctccaggggaacgtgccaccctctcctgccgtgccagtcagagtgttagcagcaatagcttagcctggtatcagcagaaacctggccaggctccccgactcctcatctatggcgcatctagccgtgccactggtatcccagaccgtttcagtggcagtgggtctgggacagacttcactctcaccatcagcagactggagcctgaagattttgcagtgtattactgtcagcagtatgagcagagccctatcacgttcggccaaggtaccaaggtggaaatcaaaggtggtggtggttcaggtggtggtggttctggcggcggctccggtggtggtggatccgaggtgcagctgttggagtctgggggaggcttggtacagcctggggggtccctgcgactctcctgtgcagcctctggattcacctttagcagctatggcatgagctgggtccgccaggctccagggaaggggctggagtgggtgtcagccattagcggtagcggtggtcagacaaattacgcagactccgtgaagggccggttcaccatctcccgtgacaattccaagaacacgctgtatctgcaaatgaacagcctgcgtgccgaggacacggctgtgtattactgtgcgagagatagaactatggggagctactactactacggtatggacgtctggggccaagggaccacggtcaccgtctcctca

SEQ ID NO: 90 - protein, 8 aa, synthetic construct
  REGION 1..8: note = Synthetic
GFTFSDYY

SEQ ID NO: 91 - protein, 8 aa, synthetic construct
  REGION 1..8: note = Synthetic
ISGSGSYT

SEQ ID NO: 92 - protein, 8 aa, synthetic construct
  REGION 1..8: note = Synthetic
AQGWAFES

SEQ ID NO: 93 - protein, 7 aa, synthetic construct
  REGION 1..7: note = Synthetic
QSVSSSY

SEQ ID NO: 94 - protein, 9 aa, synthetic construct
  REGION 1..9: note = Synthetic
QQYSRSPLT

SEQ ID NO: 95 - protein, 115 aa, synthetic construct
  REGION 1..115: note = Synthetic
EVQLLESGGGLVQPGGSLRLSCAASGFTFSDYYMSWVRQAPGKGLEWVSDISGSGSYTRYADSVKGRFTISRDNSKNTLYLQMNSLRAEDTAVYYCAQGWAFESWGQGTLVTVSS

SEQ ID NO: 96 - protein, 108 aa, synthetic construct; identical to SEQ ID NO: 70
  REGION 1..108: note = Synthetic

SEQ ID NO: 97 - protein, 242 aa, synthetic construct
  REGION 1..242: note = Synthetic
EIVLTQSPGTLSLSPGERATLSCRASQSVSSSYLAWYQQKPGQAPRLLIYGASSRATGIPDRFSGSGSGTDFTLTISRLEPEDFAVYYCQQYSRSPLTFGQGTKVEIKGGGGSGGGGSGGGSGGGGSEVQLLESGGGLVQPGGSLRLSCAASGFTFSDYYMSWVRQAPGKGLEWVSDISGSGSYTRYADSVKGRFTISRDNSKNTLYLQMNSLRAEDTAVYYCAQGWAFESWGQGTLVTVSS

SEQ ID NO: 98 - DNA, 727 bp, synthetic construct
  misc_feature 1..727: note = Synthetic
  source 1..727: mol_type = other DNA
gaaattgtgttgacgcagtctccaggcaccctgtctttgtctccaggggaacgtgccaccctctcctgccgtgccagtcagagtgttagcagcagctatttagcctggtatcagcagaaacctggccaggctccccgactcctcatctatggcgcatctagccgtgccactggtatcccagaccgtttcagtggcagtgggtctgggacagacttcactctcaccatcagcagactggagcctgaagattttgcagtgtattactgtcagcagtatagccgcagccctctgacgttcggccaaggtaccaaggtggaaatcaaaggtggtggtggttcaggtggtggtggttctggcggcggctccggtggtggtggatccgaggtgcagctgttggagtctgggggaggcttggtacagcctggggggtccctgcgactctcctgtgcagcctctggattcacctttagcgactattatatgagctgggtccgccaggctccagggaaggggctggagtgggtgtcagacattagcggtagcggtagctatacacgctacgcagactccgtgaagggccggttcaccatctcccgtgacaattccaagaacacgctgtatctgcaaatgaacagcctgcgtgccgaggacacggctgtgtattactgtgcacaaggctgggcttttgagtcctggggccagggaaccctggtcaccgtctcctcag

SEQ ID NO: 99 - protein, 14 aa, synthetic construct
  REGION 1..14: note = Synthetic
AKDIFSYLAEGMDV

SEQ ID NO: 100 - protein, 9 aa, synthetic construct
  REGION 1..9: note = Synthetic
QQYYEYPYT

SEQ ID NO: 101 - protein, 121 aa, synthetic construct
  REGION 1..121: note = Synthetic
EVQLLESGGGLVQPGGSLRLSCAASGFTFSSYGMSWVRQAPGKGLEWVSRISGYGSSTNYADSVKGRFTISRDNSKNTLYLQMNSLRAEDTAVYYCAKDIFSYLAEGMDVWGQGTTVTVSS

SEQ ID NO: 102 - protein, 108 aa, synthetic construct
  REGION 1..108: note = Synthetic
EIVLTQSPGTLSLSPGERATLSCRASQSVSSSYLAWYQQKPGQAPRLLIYGASSRATGIPDRFSGSGSGTDFTLTISRLEPEDFAVYYCQQYYEYPYTFGQGTKVEIK

SEQ ID NO: 103 - protein, 248 aa, synthetic construct
  REGION 1..248: note = Synthetic
EIVLTQSPGTLSLSPGERATLSCRASQSVSSSYLAWYQQKPGQAPRLLIYGASSRATGIPDRFSGSGSGTDFTLTISRLEPEDFAVYYCQQYYEYPYTFGQGTKVEIKGGGGSGGGGSGGGSGGGGSEVQLLESGGGLVQPGGSLRLSCAASGFTFSSYGMSWVRQAPGKGLEWVSRISGYGSSTNYADSVKGRFTISRDNSKNTLYLQMNSLRAEDTAVYYCAKDIFSYLAEGMDVWGQGTTVTVSS

SEQ ID NO: 104 - DNA, 744 bp, synthetic construct
  misc_feature 1..744: note = Synthetic
  source 1..744: mol_type = other DNA
gaaattgtgttgacgcagtctccaggcaccctgtctttgtctccaggggaacgtgccaccctctcctgccgtgccagtcagagtgttagcagcagctatttagcctggtatcagcagaaacctggccaggctccccgactcctcatctatggcgcatctagccgtgccactggtatcccagaccgtttcagtggcagtgggtctgggacagacttcactctcaccatcagcagactggagcctgaagattttgcagtgtattactgtcagcagtattatgagtatccttatacgttcggccaaggtaccaaggtggaaatcaaaggtggtggtggttcaggtggtggtggttctggcggcggctccggtggtggtggatccgaggtgcagctgttggagtctgggggaggcttggtacagcctggggggtccctgcgactctcctgtgcagcctctggattcacctttagcagctatggcatgagctgggtccgccaggctccagggaaggggctggagtgggtgtcacgcattagcggttatggtagcagcacaaattacgcagactccgtgaagggccggttcaccatctcccgtgacaattccaagaacacgctgtatctgcaaatgaacagcctgcgtgccgaggacacggctgtgtattactgtgcaaaagatatcttctcttatttggcggagggtatggacgtctggggccaagggaccacggtcaccgtctcctca

SEQ ID NO: 105 - protein, 8 aa, synthetic construct
  REGION 1..8: note = Synthetic
QASYLAWY

SEQ ID NO: 106 - protein, 8 aa, synthetic construct
  REGION 1..8: note = Synthetic
ISGSGDYT

SEQ ID NO: 107 - protein, 18 aa, synthetic construct
  REGION 1..18: note = Synthetic
ARETRQWLGLYYYYGMDV

SEQ ID NO: 108 - protein, 125 aa, synthetic construct
  REGION 1..125: note = Synthetic
TQSPGTLSLSPGERATLSCRASQSVQASYLAWYQQKPGQAPGKGLEWVSAISGSGDYTDYADSVKGRFTISRDNSKNTLYLQMNSLRAEDTAVYYCARETRQWLGLYYYYGMDVWGQGTTVTVSS

SEQ ID NO: 109 - DNA, 375 bp, synthetic construct
  misc_feature 1..375: note = Synthetic
  source 1..375: mol_type = other DNA
acgcagtctccaggcaccctgtctttgtctccaggggaacgtgccaccctctcctgccgtgccagtcagagtgttcaggccagctatttagcctggtatcagcagaaacctggccaggctccagggaaggggctggagtgggtgtcagctattagtggtagcggtgactatacagactacgcagactccgtgaagggccggttcaccatctcccgtgacaattccaagaacacgctgtatctgcaaatgaacagcctgcgtgccgaggacacggctgtgtattactgtgcgagagagacgcggcagtggctgggcctctactactactacggtatggacgtctggggccaagggaccacggtcaccgtctcctca

SEQ ID NO: 110 - protein, 19 aa, synthetic construct
  REGION 1..19: note = Synthetic
GGGGSGGGGSGGGSGGGGS

SEQ ID NO: 111 - protein, 15 aa, synthetic construct
  REGION 1..15: note = Synthetic
GGGGSGGGGSGGGGS

SEQ ID NO: 112 - protein, 24 aa, synthetic construct
  REGION 1..24: note = Synthetic
GGGGSGGGGSGGGGSGGGSGGGGS

SEQ ID NO: 113 - protein, 29 aa, synthetic construct
  REGION 1..29: note = Synthetic
GGGGSGGGGSGGGGSGGGGSGGGSGGGGS

SEQ ID NO: 114 - protein, 5 aa, synthetic construct
  REGION 1..5: note = Synthetic
GGGGS

SEQ ID NO: 115 - protein, 10 aa, synthetic construct
  REGION 1..10: note = Synthetic
GGGGSGGGGS

SEQ ID NO: 116 - protein, 335 aa, Homo sapiens
MGHPPLLPLLLLLHTCVPASWGLRCMQCKTNGDCRVEECALGQDLCRTTIVRLWEEGEELELVEKSCTHSEKTNRTLSYRTGLKITSLTEVVCGLDLCNQGNSGRAVTYSRSRYLECISCGSSDMSCERGRHQSLQCRSPEEQCLDVVTHWIQEGEEGRPKDDRHLRGCGYLPGCPGSNGFHNNDTFHFLKCCNTTKCNEGPILELENLPQNGRQCYSCKGNSTHGCSSEETFLIDCRGPMNQCLVATGTHEPKNQSYMVRGCATASMCQHAHLGDAFSMNHIDVSCCTKSGCNHPDLDVQYRSGAAPQPGPAHLSLTITLLMTARLWGGTLLWT

SEQ ID NO: 117 - protein, 235 aa, synthetic construct
  REGION 1..235: note = Synthetic
MALPVTALLLPLALLLHAARPSQFRVSPLDRTWNLGETVELKCQVLLSNPTSGCSWLFQPRGAAASPTFLLYLSQNKPKAAEGLDTQRFSGKRLGDTFVLTLSDFRRENEGYYFCSALSNSIMYFSHFVPVFLPAKPTTTPAPRPPTPAPTIASQPLSLRPEACRPAAGGAVHTRGLDFACDIYIWAPLAGTCGVLLLSLVITLYCNHRNRRRVCKCPRPVVKSGDKPSLSARYV

SEQ ID NO: 118 - protein, 247 aa, synthetic construct
  REGION 1..247: note = Synthetic
MASPLTRFLSLNLLLMGESIILGSGEAKPQAPELRIFPKKMDAELGQKVDLVCEVLGSVSQGCSWLFQNSSSKLPQPTFVVYMASSHNKITWDEKLNSSKLFSAVRDTNNKYVLTLNKFSKENEGYYFCSVISNSVMYFSSVVPVLQKVNSTTTKPVLRTPSPVHPTGTSQPQRPEDCRPRGSVKGTGLDFACDIYIWAPLAGICVAPLLSLIITLICYHRSRKRVCKCPRPLVRQEGKPRPSEKIV

SEQ ID NO: 119 - protein, 220 aa, synthetic construct
  REGION 1..220: note = Synthetic
MLRLLLALNLFPSIQVTGNKILVKQSPMLVAYDNAVNLSCKYSYNLFSREFRASLHKGLDSAVEVCVVYGNYSQQLQVYSKTGFNCDGKLGNESVTFYLQNLYVNQTDIYFCKIEVMYPPPYLDNEKSNGTIIHVKGKHLCPSPLFPGPSKPFWVLVVVGGVLACYSLLVTVAFIIFWVRSKRSRLLHSDYMNMTPRRPGPTRKHYQPYAPPRDFAAYRS

SEQ ID NO: 120 - protein, 218 aa, synthetic construct
  REGION 1..218: note = Synthetic
MTLRLLFLALNFFSVQVTENKILVKQSPLLVVDSNEVSLSCRYSYNLLAKEFRASLYKGVNSDVEVCVGNGNFTYQPQFRSNAEFNCDGDFDNETVTFRLWNLHVNHTDIYFCKIEFMYPPPYLDNERSNGTIIHIKEKHLCHTQSSPKLFWALVVVAGVLFCYGLLVTVALCVIWTNSRRNRLLQSDYMNMTPRRPGLTRKPYQPYAPARDFAAYRP

SEQ ID NO: 121 - protein, 164 aa, synthetic construct
  REGION 1..164: note = Synthetic
MKWKALFTAAILQAQLPITEAQSFGLLDPKLCYLLDGILFIYGVILTALFLRVKFSRSADAPAYQQGQNQLYNELNLGRREEYDVLDKRRGRDPEMGGKPQRRKNPQEGLYNELQKDKMAEAYSEIGMKGERRRGKGHDGLYQGLSTATKDTYDALHMQALPPR

SEQ ID NO: 122 - protein, 255 aa, synthetic construct
  REGION 1..255: note = Synthetic
MGNSCYNIVATLLLVLNFERTRSLQDPCSNCPAGTFCDNNRNQICSPCPPNSFSSAGGQRTCDICRQCKGVFRTRKECSSTSNAECDCTPGFHCLGAGCSMCEQDCKQGQELTKKGCKDCCFGTFNDQKRGICRPWTNCSLDGKSVLVNGTKERDVVCGPSPADLSPGASSVTPPAPAREPGHSPQIISFFLALTSTALLFLLFFLTLRFSVVKRGRKKLLYIFKQPFMRPVQTTQEEDGCSCRFPEEEEGGCEL

SEQ ID NO: 123 - protein, 22 aa, synthetic construct
  REGION 1..22: note = Synthetic
QNQLYNELNLGRREEYDVLDKR

SEQ ID NO: 124 - DNA, 66 bp, synthetic construct
  misc_feature 1..66: note = Synthetic
  source 1..66: mol_type = other DNA
cagaaccagctctataacgagctcaatctaggacgaagagaggagtacgatgttttggacaagaga

SEQ ID NO: 125 - protein, 22 aa, synthetic construct
  REGION 1..22: note = Synthetic
QNQLFNELNLGRREEFDVLDKR

SEQ ID NO: 126 - DNA, 66 bp, synthetic construct
  misc_feature 1..66: note = Synthetic
  source 1..66: mol_type = other DNA
cagaaccagctctttaacgagctcaatctaggacgaagagaggagttcgatgttttggacaagaga

SEQ ID NO: 127 - protein, 23 aa, synthetic construct
  REGION 1..23: note = Synthetic
QEGLYNELQKDKMAEAYSEIGMK

SEQ ID NO: 128 - DNA, 69 bp, synthetic construct
  misc_feature 1..69: note = Synthetic
  source 1..69: mol_type = other DNA
caggaaggcctgtacaatgaactgcagaaagataagatggcggaggcctacagtgagattgggatgaaa

SEQ ID NO: 129 - protein, 23 aa, synthetic construct
  REGION 1..23: note = Synthetic
QEGLFNELQKDKMAEAFSEIGMK

SEQ ID NO: 130 - DNA, 69 bp, synthetic construct
  misc_feature 1..69: note = Synthetic
  source 1..69: mol_type = other DNA
caggaaggcctgttcaatgaactgcagaaagataagatggcggaggccttcagtgagattgggatgaaa

SEQ ID NO: 131 - protein, 22 aa, synthetic construct
  REGION 1..22: note = Synthetic
HDGLYQGLSTATKDTYDALHMQ

SEQ ID NO: 132 - DNA, 66 bp, synthetic construct
  misc_feature 1..66: note = Synthetic
  source 1..66: mol_type = other DNA
cacgatggcctttaccagggtctcagtacagccaccaaggacacctacgacgcccttcacatgcag

SEQ ID NO: 133 - protein, 22 aa, synthetic construct
  REGION 1..22: note = Synthetic
HDGLFQGLSTATKDTFDALHMQ

SEQ ID NO: 134 - DNA, 66 bp, synthetic construct
  misc_feature 1..66: note = Synthetic
  source 1..66: mol_type = other DNA
cacgatggccttttccaggggctcagtacagccaccaaggacaccttcgacgcccttcacatgcag

SEQ ID NO: 135 - protein, 112 aa, synthetic construct
  REGION 1..112: note = Synthetic
RVKFSRSADAPAYQQGQNQLYNELNLGRREEYDVLDKRRGRDPEMGGKPRRKNPQEGLFNELQKDKMAEAFSEIGMKGERRRGKGHDGLFQGLSTATKDTFDALHMQALPPR

SEQ ID NO: 136 - DNA, 336 bp, synthetic construct
  misc_feature 1..336: note = Synthetic
  source 1..336: mol_type = other DNA
agagtgaagttcagcaggagcgcagacgcccccgcgtaccagcagggccagaaccagctctataacgagctcaatctaggacgaagagaggagtacgatgttttggacaagagacgtggccgggaccctgagatggggggaaagccgagaaggaagaaccctcaggaaggcctgttcaatgaactgcagaaagataagatggcggaggccttcagtgagattgggatgaaaggcgagcgccggaggggcaaggggcacgatggccttttccaggggctcagtacagccaccaaggacaccttcgacgcccttcacatgcaggccctgccccctcgc